European Patent Application EP 4 252 764 A1, published October 4, 2023. Title: Parabacteroides distasonis strain isolated from human feces and applications thereof. Applicant: GREENTECH. The sequence listing filed with the application follows.

SEQUENCE LISTING (1 sequence)

SEQ ID NO: 1 - RNA, 10653 nt, Parabacteroides distasonis
aaaggaggtgttccagccgcaccttccggtacggctaccttgttacgacttagccccagtcaccagttttaccctaggccgatcctcgcggttacggacttcaggtacccccggctcccatggcttgacgggcggtgtgtacaaggcccgggaacgtattcaccgcgccatggctgatgcgcgattactagcgaatccagcttcacggagtcgggttgcagactccgatccgaactgagacgtggtttggggattcgctccctgtcgccaggtggcctccctttgtccacgccattgtaacacgtgtgtcgccccggatgtaagggccgtgctgatttgacgtcatccccgccttcctcgcagcttacgctggcagtcccaccagagtcctcagctttacctgttagtaactagtggcaagggttgcgctcgttatggcacttaagccgacacctcacggcacgagctgacgacaaccatgcagcacctcgcaaacggctattgctagaaaaggtgtttccacctcggtccgaatgcgttcaaacccgggtaaggttcctcgcgtatcatcgaattaaaccacatgttcctccgcttgtgcgggcccccgtcaattcctttgagtttcaccgttgccggcgtactccccaggtggatcacttaacgctttcgctgtgccgcttacagtgtatcgcaaacagctagtgatcatcgtttactgcgtggactaccagggtatctaatcctgtttgatccccacgctttcgtgcatcagcgtcagtaatggcttggcaggctgccttcgcaatcggggttctgcgtgatatctatgcatttcaccgctacaccacgcattccgcctgcctcaaacatactcaagccccccagtttcaacggcaattctatggttgagccacagactttcaccgctgacttaaaaggccgcctacgcaccctttaaacccaataaatccggataacgctcggatcctccgtattaccgcggctgctggcacggagttagccgatccttattcataaggtacatacaaaacgggacacgtcccgcactttattcccttataaaagaggtttacgatccatagaaccttcatccctcacgcgacttggctggttcaggcttacgcccattgaccaatattcctcactgctgcctcccgtaggagtttggtccgtgtctcagtaccaatgtgggggaccttcctctcagaacccctatccatcgtcggtttggtgggccgttaccccgccaactgcctaatggaacgcatgcctatctatcagcgatgaatctttagcaaatatccccatgcggggcccctgcttcatgcggtattagtccgactttcgccgggttatccccctctgataggcaagttgcatacgcgttactcacccgtgcgccggtcgccggcgggtatcgctacccccgctgcccctcgacttgcatgtgttaagcctgtcgctagcgttcatcctgagccaggatcaaactcttcgaaaggaggtgttccagccgcaccttccggtacggctaccttgttacgacttagccccagtcaccagttttaccctaggccgatcctttcggttacggacttcaggtacccccggctcccatggcttgacgggcggtgtgtacaaggcccgggaacgtattcaccgcgccatggctgatgcgcgattactagcgaatccagcttcacggagtcgggttgcagactccgatccgaactgagacgtggtttggggattcgctccctgtcgccaggtggcctccctttgtccacgccattgtaacacgtgtgtcgccccggatgtaagggccgtgctgatttgacgtcatccccgccttcctcgcagcttacgctggcagtcccaccagagtcctcagctttacctgttagtaactagtggcaagggttgcgctcgttatggcacttaagccgacacctcacggcacgagctgacgacaaccatgcagcacctcgcaaacggctattgctagaaaaggtgtttccacctcggtccgaatgcgttcaaacccgggtaaggttcctcgcgtatcatcgaattaaaccacatgttcctccgcttgtgcgggcccccgtcaattcctttgagtttcaccgttgccggcgtactccccaggtggatcacttaacgctttcgctgtgccgcttacagtgtatcgcaaacagctagtgatcatcgtttactgcgtggactaccagggtatctaatcctgtttgatccccacgctttcgtgcatcagcgtcagtaatggcttggcaggctgccttcgcaatcggggttctgcgtgatatctatgcatttcaccgctacaccacgcattccgcctgcctcaaacatactcaagccccccagtttcaacggcaattctatggttgagccacagactttcaccgctgacttaaaaggccgcctacgcaccctttaaacccaataaatccggataacgctcggatcctccgtattaccgcggctgctggcacggagttagccgatccttattcataaggtacatacaaaacgggacacgtcccgcactttattcccttataaaagaggtttacgatccatagaaccttcatccctcacgcgacttggctggttcagcctctcggccattgaccaatattcctcactgctgcctcccgtaggagtttggtccgtgtctcagtaccaatgtgggggaccttcctctcagaacccctatccatcgtcggtttggtgggccgttaccccgccaactgcctaatggaacgcatgcctatctatcagcgatgaatctttagcaaatatccccatgcggggcccctgcttcatgcggtattagtccgactttcgccgggttatccccctctgataggtaagttgcatacgcgttactcacccgtgcgccggtcgccggcgggtattgctacccccgctgcccctcgacttgcatgtgttaagcctgtcgctagcgttcatcctgagccaggatcaaactcttcgcgaagagtttgatcctggctcaggatgaacgctagcgacaggcttaacacatgcaagtcgaggggcagcacaggtagcaataccgggtggcgaccggcgcacgggtgagtaacgcgtatgcaacttacctatcagagggggataacccggcgaaagtcggactaataccgcatgaagcaggggtcccgcatggggatatttgctaaagattcatcgctgatagataggcatgcgttccattaggcagttggcggggtaacggcccaccaaaccgacgatggataggggttctgagaggaaggtcccccacattggtactgagacacggaccaaactcctacgggaggcagcagtgaggaatattggtcaatggccgagaggctgaaccagccaagtcgcgtgagggatgaaggttctatggatcgtaaacctcttttataagggaataaagtgcgggacgtgtcccgttttgtatgtaccttatgaataaggatcggctaactccgtgccagcagccgcggtaatacggaggatccgagcgttatccggatttattgggtttaaagggtgcgtaggcggccttttaagtcagcggtgaaagtctgtggctcaaccatagaattgccgttgaaactggggggcttgagtatgtttgaggcaggcggaatgcgtggtgtagcggtgaaatgcatagatatcacgcagaaccccgattgcgaaggcagcctgccaagccattactgacgctgatgcacgaaagcgtggggatcaaacaggattagataccctggtagtccacgcagtaaacgatgatcactagctgtttgcgatacactgtaagcggcacagcgaaagcgttaagtgatccacctggggagtacgccggcaacggtgaaactcaaaggaattgacgggggcccgcacaagcggaggaacatgtggtttaattcgatgatacgcgaggaaccttacccgggtttgaacgcattcggaccgaggtggaaacaccttttctagcaatagccgtttgcgaggtgctgcatggttgtcgtcagctcgtgccgtgaggtgtcggcttaagtgccataacgagcgcaacccttgccactagttactaacaggtaaagctgaggactctggtgggactgccagcgtaagctgcgaggaaggcggggatgacgtcaaatcagcacggcccttacatccggggcgacacacgtgttacaatggcgtggacaaagggaagccacctggcgacagggagcgaatccccaaaccacgtctcagttcggatcggagtctgcaacccgactccgtgaagctggattcgctagtaatcgcgcatcagccatggcgcggtgaatacgttcccgggccttgtacacaccgcccgtcaagccatgggagccgggggtacctgaagtccgtaactgcgaggatcggcctagggtaaaactggtgactggggctaagtcgtaacaaggtagccgtaccggaaggtgcggctggaacacctcctttcgaagagtttgatcctggctcaggatgaacgctagcgacaggcttaacacatgcaagtcgaggggcagcacaggtagcaataccgggtggcgaccggcgcacgggtgagtaacgcgtatgcaacttacctatcagagggggataacccggcgaaagtcggactaataccgcatgaagcaggggtcccgcatggggatatttgctaaagattcatcgctgatagataggcatgcgttccattaggcagttggcggggtaacggcccaccaaaccgacgatggataggggttctgagaggaaggtcccccacattggtactgagacacggaccaaactcctacgggaggcagcagtgaggaatattggtcaatggccgagaggctgaaccagccaagtcgcgtgagggatgaaggttctatggatcgtaaacctcttttataagggaataaagtgcgggacgtgtcccgttttgtatgtaccttatgaataaggatcggctaactccgtgccagcagccgcggtaatacggaggatccgagcgttatccggatttattgggtttaaagggtgcgtaggcggccttttaagtcagcggtgaaagtctgtggctcaaccatagaattgccgttgaaactggggggcttgagtatgtttgaggcaggcggaatgcgtggtgtagcggtgaaatgcatagatatcacgcagaaccccgattgcgaaggcagcctgccaagccattactgacgctgatgcacgaaagcgtggggatcaaacaggattagataccctggtagtccacgcagtaaacgatgatcactagctgtttgcgatacactgtaagcggcacagcgaaagcgttaagtgatccacctggggagtacgccggcaacggtgaaactcaaaggaattgacgggggcccgcacaagcggaggaacatgtggtttaattcgatgatacgcgaggaaccttacccgggtttgaacgcattcggaccgaggtggaaacaccttttctagcaatagccgtttgcgaggtgctgcatggttgtcgtcagctcgtgccgtgaggtgtcggcttaagtgccataacgagcgcaacccttgccactagttactaacaggtaaagctgaggactctggtgggactgccagcgtaagctgcgaggaaggcggggatgacgtcaaatcagcacggcccttacatccggggcgacacacgtgttacaatggcgtggacaaagggaagccacctggcgacagggagcgaatccccaaaccacgtctcagttcggatcggagtctgcaacccgactccgtgaagctggattcgctagtaatcgcgcatcagccatggcgcggtgaatacgttcccgggccttgtacacaccgcccgtcaagccatgggagccgggggtacctgaagtccgtaaccgcgaggatcggcctagggtaaaactggtgactggggctaagtcgtaacaaggtagccgtaccggaaggtgcggctggaacacctcctttcgaagagtttgatcctggctcaggatgaacgctagcgacaggcttaacacatgcaagtcgaggggcagcacaggtagcaataccgggtggcgaccggcgcacgggtgagtaacgcgtatgcaacttacctatcagagggggataacccggcgaaagtcggactaataccgcatgaagcaggggtcccgcatggggatatttgctaaagattcatcgctgatagataggcatgcgttccattaggcagttggcggggtaacggcccaccaaaccgacgatggatagggggcctagttctgagaggaaggtcccccacattggtactgagacacggaccaaactcctacgggaggcagcagtgaggaatattggtcaatggccgagaggctgaaccagccaagtcgcgtgagggatgaaggttctatggatcgtaaacctcttttataagggaataaagtgcgggacgtgtcccgttttgtatgtaccttatgaataaggatcggctaactccgtgccagcagccgcggtaatacggaggatccgagcgttatccggatttattgggtttaaagggtgcgtaggcggccttttaagtcagcggtgaaagtctgtggctcaaccatagaattgccgttgaaactggggggcttgagtatgtttgaggcaggcggaatgcgtggtgtagcggtgaaatgcatagatatcacgcagaaccccgattgcgaaggcagcctgccaagccattactgacgctgatgcacgaaagcgtggggatcaaacaggattagataccctggtagtccacgcagtaaacgatgatcactagctgtttgcgatacactgtaagcggcacagcgaaagcgttaagtgatccacctggggagtacgccggcaacggtgaaactcaaaggaattgacgggggcccgcacaagcggaggaacatgtggtttaattcgatgatacgcgaggaaccttacccgggtttgaacgcattcggaccgaggtggaaacaccttttctagcaatagccgtttgcgaggtgctgcatggttgtcgtcagctcgtgccgtgaggtgtcggcttaagtgccataacgagcgcaacccttgccactagttactaacaggtaaagctgaggactctggtgggactgccagcgtaagctgcgaggaaggcggggatgacgtcaaatcagcacggcccttacatccggggcgacacacgtgttacaatggcgtggacaaagggaagccacctggcgacagggagcgaatccccaaaccacgtctcagttcggatcggagtctgcaacccgactccgtgaagctggattcgctagtaatcgcgcatcagccatggcgcggtgaatacgttcccgggccttgtacacaccgcccgtcaagccatgggagccgggggtacctgaagtccgtaactgcgaggatcggcctagggtaaaactggtgactggggctaagtcgtaacaaggtagccgtaccggaaggtgcggctggaacacctcctttaaaggaggtgttccagccgcaccttccggtacggctaccttgttacgacttagccccagtcaccagttttaccctaggccgatcctttcggttacggacttcaggtacccccggctcccatggcttgacgggcggtgtgtacaaggcccgggaacgtattcaccgcgccatggctgatgcgcgattactagcgaatccagcttcacggagtcgggttgcagactccgatccgaactgagacgtggtttggggattcgctccctgtcgccaggtggcctccctttgtccacgccattgtaacacgtgtgtcgccccggatgtaagggccgtgctgatttgacgtcatccccgccttcctcgcagcttacgctggcagtcccaccagagtcctcagctttacctgttagtaactagtggcaagggttgcgctcgttatggcacttaagccgacacctcacggcacgagctgacgacaaccatgcagcacctcgcaaacggctattgctagaaaaggtgtttccacctcggtccgaatgcgttcaaacccgggtaaggttcctcgcgtatcatcgaattaaaccacatgttcctccgcttgtgcgggcccccgtcaattcctttgagtttcaccgttgccggcgtactccccaggtggatcacttaacgctttcgctgtgccgcttacagtgtatcgcaaacagctagtgatcatcgtttactgcgtggactaccagggtatctaatcctgtttgatccccacgctttcgtgcatcagcgtcagtaatggcttggcaggctgccttcgcaatcggggttctgcgtgatatctatgcatttcaccgctacaccacgcattccgcctgcctcaaacatactcaagccccccagtttcaacggcaattctatggttgagccacagactttcaccgctgacttaaaaggccgcctacgcaccctttaaacccaataaatccggataacgctcggatcctccgtattaccgcggctgctggcacggagttagccgatccttattcataaggtacatacaaaacgggacacgtcccgcactttattcccttataaaagaggtttacgatccatagaaccttcatccctcacgcgacttggctggttcaggcttacgcccattgaccaatattcctcactgctgcctcccgtaggagtttggtccgtgtctcagtaccaatgtgggggaccttcctctcagaacccctatccatcgtcggtttggtgggccgttaccccgccaactgcctaatggaacgcatgcctatctatcagcgatgaatctttagcaaatatccccatgcggggcccctgcttcatgcggtattagtccgactttcgccgggttatccccctctgataggcaagttgcatacgcgttactcacccgtgcgccggtcgccggcgggtatcgctacccccgctgcccctcgacttgcatgtgttaagcctgtcgctagcgttcatcctgagccaggatcaaactcttcgaaaggaggtgttccagccgcaccttccggtacggctaccttgttacgacttagccccagtcaccagttttaccctaggccgatcctcgcggttacggacttcaggtacccccggctcccatggcttgacgggcggtgtgtacaaggcccgggaacgtattcaccgcgccatggctgatgcgcgattactagcgaatccagcttcacggagtcgggttgcagactccgatccgaactgagacgtggtttggggattcgctccctgtcgccaggtggcttccctttgtccacgccattgtaacacgtgtgtcgccccggatgtaagggccgtgctgatttgacgtcatccccgccttcctcgcagcttacgctggcagtcccaccagagtcctcagctttacctgttagtaactagtggcaagggttgcgctcgttatggcacttaagccgacacctcacggcacgagctgacgacaaccatgcagcacctcgcaaacggctattgctagaaaaggtgtttccacctcggtccgaatgcgttcaaacccgggtaaggttcctcgcgtatcatcgaattaaaccacatgttcctccgcttgtgcgggcccccgtcaattcctttgagtttcaccgttgccggcgtactccccaggtggatcacttaacgctttcgctgtgccgcttacagtgtatcgcaaacagctagtgatcatcgtttactgcgtggactaccagggtatctaatcctgtttgatccccacgctttcgtgcatcagcgtcagtaatggcttggcaggctgccttcgcaatcggggttctgcgtgatatctatgcatttcaccgctacaccacgcattccgcctgcctcaaacatactcaagccccccagtttcaacggcaattctatggttgagccacagactttcaccgctgacttaaaaggccgcctacgcaccctttaaacccaataaatccggataacgctcggatcctccgtattaccgcggctgctggcacggagttagccgatccttattcataaggtacatacaaaacgggacacgtcccgcactttattcccttataaaagaggtttacgatccatagaaccttcatccctcacgcgacttggctggttcagcctctcggccattgaccaatattcctcactgctgcctcccgtaggagtttggtccgtgtctcagtaccaatgtgggggaccttcctctcagaacccctatccatcgtcggtttggtgggccgttaccccgccaactgcctaatggaacgcatgcctatctatcagcgatgaatctttagcaaatatccccatgcgggatccctgcttcatgcggtattagtccgactttcgccgggttatccccctctgataggcaagttgcatacgcgttactcacccgtgcgccggtcgccacccggtattgctacctgtgctgcccctcgacttgcatgtgttaagcctgtcgctagcgttcatcctgagccaggatcaaactcttcg